European Patent Application EP 4 541 884 A1, published April 23, 2025. Title: MODIFIED XYLOSE REDUCTASE AND USES THEREOF. Applicant: Annikki GmbH. The sequence listing filed with the application follows.

SEQUENCE LISTING (30 sequences)

SEQ ID NO: 1 - protein, 329 aa, Kluyveromyces marxianus
MTYLAPTVTLNNGSKMPLVGLGCWKIPNEVCAEQVYEAIKLGYRLFDGAQDYANEKEVGQGINRAIKEGIVKREDLVVVSKLWNSFHHPDNVRTAVERTLNDLQLDYLDLFYIHFPLAFKFVPLDEKYPPGFYTGKDNFAKEIIEEEPVPILDTYRALEKLVDEGLIKSLGISNFSGALIQDLLRGARIKPVALQIEHHPYLVQDRLITYAQKVGLQVVAYSSFGPLSFVELNNEKALHTKTLFENDTIKAIAQKHNVTPSHVLLKWSTQRGIAVIPKSSKKERLLENLKIEETFTLSDEEIKEINGLDQGLRFNDPWDWLGNEFPTFI

SEQ ID NO: 2 - protein, 322 aa, Chaetomium globosum
MAPVIKLNSGYDMPQVGFGLWKVDNAVASDVVYNAIKAGYRLFDGACDYGNEVECGQGVARAISEGIVKREDLFIVSKLWNTFHDAERVEPIVKKQLADWGIEYFDLYLIHFPVALEWVDPAVRYPPGWHYDGKEEIRPSKATIQETWTALESLVSKGLSKSIGISNFQAQLIYDLLRYAKIRPATLQVEHHPYLVQQELINLAKREGIAVTAYSSFGPASFKEFNMKHADALAPLIEDETIKKIAAKHNRPASQVLLRWATQRGLAIIPKSTRPQIMAENFQSIDFDLSEEDIATISAFDRGIRFNQPSNYFPTELLWIFG

SEQ ID NO: 3 - protein, 317 aa, Candida parapsilosis
MSIKLNSGHEMPIVGFGCWKVTNETAADQIYNAIKVGYRLFDGAQDYGNEKEVGEGINRAIDEGLVSRDELFVVSKLWNNYHDPKNVETALNKTLSDLNLEYLDLFLIHFPIAFKFVPIEEKYPPGFYCGDGDKFHYENVPLLDTWRALESLVQKGKIRSIGISNFNGGLIYDLVRGAKIKPAVLQIEHHPYLQQPRLIEFVQSQGIAITGYSSFGPQSFLELESKKALDTPTLFDHETIKSIASKHKKSSAQVLLRWATQRGIAVIPKSNNPDRLAQNLNVSDFELSKEDLEAINKLDKGLRFNDPWDWDHIPIFV

SEQ ID NO: 4 - protein, 324 aa, Candida tropicalis
MSTTVNTPTIKLNSGYEMPLVGFGCWKVTNATAADQIYNAIKTGYRLFDGAEDYGNEKEVGEGINRAIKDGLVKREELFITSKLWNNFHDPKNVETALNKTLSDLNLDYVDLFLIHFPIAFKFVPIEEKYPPGFYCGDGDNFHYEDVPLLDTWKALEKLVEAGKIKSIGISNFTGALIYDLIRGATIKPAVLQIEHHPYLQQPKLIEYVQKAGIAITGYSSFGPQSFLELESKRALNTPTLFEHETIKSIADKHGKSPAQVLLRWATQRNIAVIPKSNNPERLAQNLSVVDFDLTKDDLDNIAKLDIGLRFNDPWDWDNIPIFV

SEQ ID NO: 5 - protein, 322 aa, Candida tenuis
MSASIPDIKLSSGHLMPSIGFGCWKLANATAGEQVYQAIKAGYRLFDGAEDYGNEKEVGDGVKRAIDEGLVKREEIFLTSKLWNNYHDPKNVETALNKTLADLKVDYVDLFLIHFPIAFKFVPIEEKYPPGFYCGDGNNFVYEDVPILETWKALEKLVAAGKIKSIGVSNFPGALLLDLLRGATIKPAVLQVEHHPYLQQPKLIEFAQKAGVTITAYSSFGPQSFVEMNQGRALNTPTLFAHDTIKAIAAKYNKTPAEVLLRWAAQRGIAVIPKSNLPERLVQNRSFNTFDLTKEDFEEIAKLDIGLRFNDPWDWDNIPIFV

SEQ ID NO: 6 - DNA, 990 bp, Kluyveromyces marxianus
  source 1..990: mol_type = genomic DNA
atgacatacctcgcaccaacagttaccttgaacaatggatccaagatgccgctagtcggcttgggatgctggaaaatcccaaacgaagtgtgtgccgaacaggtgtacgaagccatcaagttgggctaccgcttgttcgacggcgcgcaggactacgccaacgaaaaagaggtgggccaaggtattaacagagccatcaaggaaggaatcgtcaagagagaagacttggtcgtcgtttctaagttgtggaacagtttccaccacccagacaacgtgcgtaccgcagtcgaaagaactttgaacgacttgcaattggactacttggacttgttctacatccatttcccattggctttcaagttcgtgccactagacgagaagtaccctccaggtttctacacaggtaaggacaatttcgccaaggaaatcatcgaagaggagcctgtcccaatcttggacacctacagagcccttgagaagttggtcgacgaaggtttgatcaaatctttgggtatctcaaacttttcgggtgcattgatccaggacttgttgcgtggcgcccgtatcaagccagtcgccttgcagatcgaacaccacccatacttggtccaggaccgcttgatcacgtacgcccaaaaggtgggcttgcaagtcgtcgcctactccagtttcggcccactatcctttgtcgagttgaacaacgaaaaggccttgcacacaaagactttgttcgaaaacgacaccatcaaggccatcgctcaaaaacacaacgtcaccccatcccacgtcttgttgaagtggtccacccaacgtggtatcgccgtcattccaaagtcctccaagaaggaacgtctcctcgagaacttgaagatcgaagagacctttaccttgtccgacgaagagatcaaggagatcaacggcttggaccagggattgagatttaacgacccatgggactggttgggcaacgaattcccaacctttatctaa

SEQ ID NO: 7 - DNA, 969 bp, Chaetomium globosum
  source 1..969: mol_type = genomic DNA
atggcgccggtgattaaactgaacagcggctatgatatgccgcaggtgggctttggcctgtggaaagtggataacgcggtggcgagcgatgtggtgtataacgcgattaaagcgggctatcgcctgtttgatggcgcgtgcgattatggcaacgaagtggaatgcggccagggcgtggcgcgcgcgattagcgaaggcattgtgaaacgcgaagatctgtttattgtgagcaaactgtggaacacctttcatgatgcggaacgcgtggaaccgattgtgaaaaaacagctggcggattggggcattgaatattttgatctgtatctgattcattttccggtggcgctggaatgggtggatccggcggtgcgctatccgccgggctggcattatgatggcaaagaagaaattcgcccgagcaaagcgaccattcaggaaacctggaccgcgctggaaagcctggtgagcaaaggcctgagcaaaagcattggcattagcaactttcaggcgcagctgatttatgatctgctgcgctatgcgaaaattcgcccggcgaccctgcaggtggaacatcatccgtatctggtgcagcaggaactgattaacctggcgaaacgcgaaggcattgcggtgaccgcgtatagcagctttggcccggcgagctttaaagaatttaacatgaaacatgcggatgcgctggcgccgctgattgaagatgaaaccattaaaaaaattgcggcgaaacataaccgcccggcgagccaggtgctgctgcgctgggcgacccagcgcggcctggcgattattccgaaaagcacccgcccgcagattatggcggaaaactttcagagcattgattttgatctgagcgaagaagatattgcgaccattagcgcgtttgatcgcggcattcgctttaaccagccgagcaactattttccgaccgaactgctgtggatttttggctaa

SEQ ID NO: 8 - DNA, 954 bp, Candida parapsilosis
  source 1..954: mol_type = genomic DNA
atgtccattaagctgaatagcggtcacgagatgccaattgtgggttttggttgttggaaggtgaccaatgaaaccgcggccgatcaaatttataacgcgatcaaggtcggctaccgcttgttcgacggcgcccaagactacggcaacgagaaagaggttggcgagggcatcaaccgcgcgatcgatgagggtctggtgtctcgtgacgagctgttcgttgtcagcaagctgtggaataactatcacgacccgaagaatgtcgaaacggccctgaataaaacgctgagcgatttgaacctggaatacctggatctgttcctgatccactttccgatcgcgttcaaatttgtcccgatcgaagagaaataccctccgggcttttactgcggcgatggtgataaatttcactatgaaaacgttccgctgctggacacctggcgcgccttggaaagcctggtgcagaagggtaaaatccgttccattggtatcagcaatttcaacggtggcctgatttacgatctggttcgtggcgcaaagatcaagccggctgtgctgcagattgagcatcacccgtatctgcaacagcctcgcctgattgagttcgtccagagccagggtattgcaatcaccggttattctagcttcggtccacagagcttcctggagttggaaagcaagaaagcgctggataccccgaccctgttcgaccacgaaacgattaaatccatcgctagcaaacataagaagagcagcgcacaggtgctgctgcgttgggcgactcaacgtggtattgcggttattccgaaaagcaacaatccggaccgtctggcacaaaacctgaatgttagcgactttgagttgtcgaaagaggacctggaagcgatcaacaagctggataaaggtctgcgttttaatgacccgtgggactgggatcatattccaatctttgtttaa

SEQ ID NO: 9 - DNA, 974 bp, Candida tropicalis
  source 1..974: mol_type = genomic DNA
atgagcacgaccgttaatactccgacgatcaaactgaactccggttacgagatgccgctggttggctttggctgttggaaagttaccaatgcgacggcggcggaccagatttataacgctattaaaaccggttaccgtctgttcgatggcgcagaggactacggtaacgagaaagaagtgggtgaaggtattaatcgcgcaattaaagacggtctggtcaaacgtgaagagctgtttattacctcgaaactgtggaataacttccatgatcctaagaacgtggagactgcgctgaataagaccctgagcgatctgaacctggactatgtggatctgtttctgattcacttcccgattgctttcaaatttgtcccgatcgaagaaaagtacccaccgggcttctactgcggtgacggcgacaacttccattatgaggatgttccgctgctggacacgtggaaggcgctggagaaattggtggaagccggtaagatcaagtccattggcattagcaacttcaccggtgccttgatttacgatttgatccgtggtgcgaccattaaaccggcggttctgcagatcgagcatcacccgtatctgcaacagccgaaactgatcgaatacgttcagaaagcaggtatcgccatcactggctatagcagcttcggtccacagagcttcctggagctggagagcaagcgtgccctgaataccccgacgttgtttgaacacgaaaccatcaagtctatcgctgacaaacacggtaagagccctgcacaagtcctgctgcgctgggcaacgcaacgtaatattgcggttattccgaagagcaataacccggagcgtctggcgcagaatctgtctgtcgtcgactttgatttgaccaaggatgacctggataatatcgcgaagctggacatcggcctgcgcttcaacgatccgtgggattgggacaacatcccgatctttgtgta

SEQ ID NO: 10 - DNA, 969 bp, Candida tenuis
  source 1..969: mol_type = genomic DNA
atgagcgcaagtatcccagacatcaaattgagctccggccacttaatgccttccatcggtttcggctgttggaagctcgccaacgctaccgccggtgaacaagtctaccaagccatcaaggccggttacagattgttcgacggtgccgaggactacggtaacgaaaaggaagtcggtgacggtgtcaagagagccatcgacgaaggtcttgtcaagagagaagagatcttcctcacctccaagttgtggaacaactaccacgacccaaagaacgtcgagaccgccttgaacaaaaccctcgccgaccttaaggttgactacgttgacttgttcttgatccatttcccaattgccttcaagttcgtcccaatcgaggagaagtacccaccaggattctactgtggtgacggtaacaacttcgtctacgaagacgttccaatcttggagacctggaaggccctcgagaagttggttgctgccggtaagattaagtccatcggtgtctctaacttcccaggtgctttgctcttggacttgctcagaggtgctaccatcaagccagctgtcttgcaagttgagcaccacccatacttgcaacaaccaaagttgatcgagttcgctcaaaaggccggtgttaccatcaccgcctactcttctttcggtcctcaatctttcgttgagatgaaccaaggtagagctttgaacaccccaaccttgttcgcacacgacaccatcaaggctattgctgccaagtacaacaagaccccagctgaggttttattgagatgggccgcccaaagaggtatcgctgtcattccaaagtctaacctcccagagagattagtccaaaacagaagtttcaacaccttcgacttgaccaaggaggacttcgaggaaatcgccaagttggacatcggcttgagattcaacgacccatgggactgggacaacattccaatcttcgtttaa

SEQ ID NO: 11 - protein, 324 aa, synthetic construct
  source 1..324: note = CtropXR W26Y
MSTTVNTPTIKLNSGYEMPLVGFGCYKVTNATAADQIYNAIKTGYRLFDGAEDYGNEKEVGEGINRAIKDGLVKREELFITSKLWNNFHDPKNVETALNKTLSDLNLDYVDLFLIHFPIAFKFVPIEEKYPPGFYCGDGDNFHYEDVPLLDTWKALEKLVEAGKIKSIGISNFTGALIYDLIRGATIKPAVLQIEHHPYLQQPKLIEYVQKAGIAITGYSSFGPQSFLELESKRALNTPTLFEHETIKSIADKHGKSPAQVLLRWATQRNIAVIPKSNNPERLAQNLSVVDFDLTKDDLDNIAKLDIGLRFNDPWDWDNIPIFV

SEQ ID NO: 12 - protein, 329 aa, synthetic construct
  source 1..329: note = KlmXR W24Y
MTYLAPTVTLNNGSKMPLVGLGCYKIPNEVCAEQVYEAIKLGYRLFDGAQDYANEKEVGQGINRAIKEGIVKREDLVVVSKLWNSFHHPDNVRTAVERTLNDLQLDYLDLFYIHFPLAFKFVPLDEKYPPGFYTGKDNFAKEIIEEEPVPILDTYRALEKLVDEGLIKSLGISNFSGALIQDLLRGARIKPVALQIEHHPYLVQDRLITYAQKVGLQVVAYSSFGPLSFVELNNEKALHTKTLFENDTIKAIAQKHNVTPSHVLLKWSTQRGIAVIPKSSKKERLLENLKIEETFTLSDEEIKEINGLDQGLRFNDPWDWLGNEFPTFI

SEQ ID NO: 13 - protein, 329 aa, synthetic construct
  source 1..329: note = KlmXR C23T W24F
MTYLAPTVTLNNGSKMPLVGLGTFKIPNEVCAEQVYEAIKLGYRLFDGAQDYANEKEVGQGINRAIKEGIVKREDLVVVSKLWNSFHHPDNVRTAVERTLNDLQLDYLDLFYIHFPLAFKFVPLDEKYPPGFYTGKDNFAKEIIEEEPVPILDTYRALEKLVDEGLIKSLGISNFSGALIQDLLRGARIKPVALQIEHHPYLVQDRLITYAQKVGLQVVAYSSFGPLSFVELNNEKALHTKTLFENDTIKAIAQKHNVTPSHVLLKWSTQRGIAVIPKSSKKERLLENLKIEETFTLSDEEIKEINGLDQGLRFNDPWDWLGNEFPTFI

SEQ ID NO: 14 - protein, 322 aa, synthetic construct
  source 1..322: note = CgXR W21Y
MAPVIKLNSGYDMPQVGFGLYKVDNAVASDVVYNAIKAGYRLFDGACDYGNEVECGQGVARAISEGIVKREDLFIVSKLWNTFHDAERVEPIVKKQLADWGIEYFDLYLIHFPVALEWVDPAVRYPPGWHYDGKEEIRPSKATIQETWTALESLVSKGLSKSIGISNFQAQLIYDLLRYAKIRPATLQVEHHPYLVQQELINLAKREGIAVTAYSSFGPASFKEFNMKHADALAPLIEDETIKKIAAKHNRPASQVLLRWATQRGLAIIPKSTRPQIMAENFQSIDFDLSEEDIATISAFDRGIRFNQPSNYFPTELLWIFG

SEQ ID NO: 15 - protein, 317 aa, synthetic construct
  source 1..317: note = CpXR C18T W19F
MSIKLNSGHEMPIVGFGTFKVTNETAADQIYNAIKVGYRLFDGAQDYGNEKEVGEGINRAIDEGLVSRDELFVVSKLWNNYHDPKNVETALNKTLSDLNLEYLDLFLIHFPIAFKFVPIEEKYPPGFYCGDGDKFHYENVPLLDTWRALESLVQKGKIRSIGISNFNGGLIYDLVRGAKIKPAVLQIEHHPYLQQPRLIEFVQSQGIAITGYSSFGPQSFLELESKKALDTPTLFDHETIKSIASKHKKSSAQVLLRWATQRGIAVIPKSNNPDRLAQNLNVSDFELSKEDLEAINKLDKGLRFNDPWDWDHIPIFV

SEQ ID NO: 16 - protein, 329 aa, synthetic construct
  source 1..329: note = KlmXR C23T W24F K25R
MTYLAPTVTLNNGSKMPLVGLGTFRIPNEVCAEQVYEAIKLGYRLFDGAQDYANEKEVGQGINRAIKEGIVKREDLVVVSKLWNSFHHPDNVRTAVERTLNDLQLDYLDLFYIHFPLAFKFVPLDEKYPPGFYTGKDNFAKEIIEEEPVPILDTYRALEKLVDEGLIKSLGISNFSGALIQDLLRGARIKPVALQIEHHPYLVQDRLITYAQKVGLQVVAYSSFGPLSFVELNNEKALHTKTLFENDTIKAIAQKHNVTPSHVLLKWSTQRGIAVIPKSSKKERLLENLKIEETFTLSDEEIKEINGLDQGLRFNDPWDWLGNEFPTFI

SEQ ID NO: 17 - protein, 329 aa, synthetic construct
  source 1..329: note = KlmXR C23V W24F
MTYLAPTVTLNNGSKMPLVGLGVFKIPNEVCAEQVYEAIKLGYRLFDGAQDYANEKEVGQGINRAIKEGIVKREDLVVVSKLWNSFHHPDNVRTAVERTLNDLQLDYLDLFYIHFPLAFKFVPLDEKYPPGFYTGKDNFAKEIIEEEPVPILDTYRALEKLVDEGLIKSLGISNFSGALIQDLLRGARIKPVALQIEHHPYLVQDRLITYAQKVGLQVVAYSSFGPLSFVELNNEKALHTKTLFENDTIKAIAQKHNVTPSHVLLKWSTQRGIAVIPKSSKKERLLENLKIEETFTLSDEEIKEINGLDQGLRFNDPWDWLGNEFPTFI

SEQ ID NO: 18 - protein, 329 aa, synthetic construct
  source 1..329: note = KlmXR C23L W24F
MTYLAPTVTLNNGSKMPLVGLGLFKIPNEVCAEQVYEAIKLGYRLFDGAQDYANEKEVGQGINRAIKEGIVKREDLVVVSKLWNSFHHPDNVRTAVERTLNDLQLDYLDLFYIHFPLAFKFVPLDEKYPPGFYTGKDNFAKEIIEEEPVPILDTYRALEKLVDEGLIKSLGISNFSGALIQDLLRGARIKPVALQIEHHPYLVQDRLITYAQKVGLQVVAYSSFGPLSFVELNNEKALHTKTLFENDTIKAIAQKHNVTPSHVLLKWSTQRGIAVIPKSSKKERLLENLKIEETFTLSDEEIKEINGLDQGLRFNDPWDWLGNEFPTFI

SEQ ID NO: 19 - protein, 329 aa, synthetic construct
  source 1..329: note = KlmXR C23S W24F
MTYLAPTVTLNNGSKMPLVGLGSFKIPNEVCAEQVYEAIKLGYRLFDGAQDYANEKEVGQGINRAIKEGIVKREDLVVVSKLWNSFHHPDNVRTAVERTLNDLQLDYLDLFYIHFPLAFKFVPLDEKYPPGFYTGKDNFAKEIIEEEPVPILDTYRALEKLVDEGLIKSLGISNFSGALIQDLLRGARIKPVALQIEHHPYLVQDRLITYAQKVGLQVVAYSSFGPLSFVELNNEKALHTKTLFENDTIKAIAQKHNVTPSHVLLKWSTQRGIAVIPKSSKKERLLENLKIEETFTLSDEEIKEINGLDQGLRFNDPWDWLGNEFPTFI

SEQ ID NO: 20 - protein, 329 aa, synthetic construct
  source 1..329: note = KlmXR C23I W24F
MTYLAPTVTLNNGSKMPLVGLGIFKIPNEVCAEQVYEAIKLGYRLFDGAQDYANEKEVGQGINRAIKEGIVKREDLVVVSKLWNSFHHPDNVRTAVERTLNDLQLDYLDLFYIHFPLAFKFVPLDEKYPPGFYTGKDNFAKEIIEEEPVPILDTYRALEKLVDEGLIKSLGISNFSGALIQDLLRGARIKPVALQIEHHPYLVQDRLITYAQKVGLQVVAYSSFGPLSFVELNNEKALHTKTLFENDTIKAIAQKHNVTPSHVLLKWSTQRGIAVIPKSSKKERLLENLKIEETFTLSDEEIKEINGLDQGLRFNDPWDWLGNEFPTFI

SEQ ID NO: 21 - protein, 329 aa, synthetic construct
  source 1..329: note = KlmXR C23M W24F
MTYLAPTVTLNNGSKMPLVGLGMFKIPNEVCAEQVYEAIKLGYRLFDGAQDYANEKEVGQGINRAIKEGIVKREDLVVVSKLWNSFHHPDNVRTAVERTLNDLQLDYLDLFYIHFPLAFKFVPLDEKYPPGFYTGKDNFAKEIIEEEPVPILDTYRALEKLVDEGLIKSLGISNFSGALIQDLLRGARIKPVALQIEHHPYLVQDRLITYAQKVGLQVVAYSSFGPLSFVELNNEKALHTKTLFENDTIKAIAQKHNVTPSHVLLKWSTQRGIAVIPKSSKKERLLENLKIEETFTLSDEEIKEINGLDQGLRFNDPWDWLGNEFPTFI

SEQ ID NO: 22 - protein, 329 aa, synthetic construct
  source 1..329: note = KlmXR W24F
MTYLAPTVTLNNGSKMPLVGLGCFKIPNEVCAEQVYEAIKLGYRLFDGAQDYANEKEVGQGINRAIKEGIVKREDLVVVSKLWNSFHHPDNVRTAVERTLNDLQLDYLDLFYIHFPLAFKFVPLDEKYPPGFYTGKDNFAKEIIEEEPVPILDTYRALEKLVDEGLIKSLGISNFSGALIQDLLRGARIKPVALQIEHHPYLVQDRLITYAQKVGLQVVAYSSFGPLSFVELNNEKALHTKTLFENDTIKAIAQKHNVTPSHVLLKWSTQRGIAVIPKSSKKERLLENLKIEETFTLSDEEIKEINGLDQGLRFNDPWDWLGNEFPTFI

SEQ ID NO: 23 - protein, 329 aa, synthetic construct
  source 1..329: note = KlmXR C23G W24F
MTYLAPTVTLNNGSKMPLVGLGGFKIPNEVCAEQVYEAIKLGYRLFDGAQDYANEKEVGQGINRAIKEGIVKREDLVVVSKLWNSFHHPDNVRTAVERTLNDLQLDYLDLFYIHFPLAFKFVPLDEKYPPGFYTGKDNFAKEIIEEEPVPILDTYRALEKLVDEGLIKSLGISNFSGALIQDLLRGARIKPVALQIEHHPYLVQDRLITYAQKVGLQVVAYSSFGPLSFVELNNEKALHTKTLFENDTIKAIAQKHNVTPSHVLLKWSTQRGIAVIPKSSKKERLLENLKIEETFTLSDEEIKEINGLDQGLRFNDPWDWLGNEFPTFI

SEQ ID NO: 24 - protein, 329 aa, synthetic construct
  source 1..329: note = KlmXR C23P W24F
MTYLAPTVTLNNGSKMPLVGLGPFKIPNEVCAEQVYEAIKLGYRLFDGAQDYANEKEVGQGINRAIKEGIVKREDLVVVSKLWNSFHHPDNVRTAVERTLNDLQLDYLDLFYIHFPLAFKFVPLDEKYPPGFYTGKDNFAKEIIEEEPVPILDTYRALEKLVDEGLIKSLGISNFSGALIQDLLRGARIKPVALQIEHHPYLVQDRLITYAQKVGLQVVAYSSFGPLSFVELNNEKALHTKTLFENDTIKAIAQKHNVTPSHVLLKWSTQRGIAVIPKSSKKERLLENLKIEETFTLSDEEIKEINGLDQGLRFNDPWDWLGNEFPTFI

SEQ ID NO: 25 - protein, 329 aa, synthetic construct
  source 1..329: note = KlmXR C23A W24F
MTYLAPTVTLNNGSKMPLVGLGAFKIPNEVCAEQVYEAIKLGYRLFDGAQDYANEKEVGQGINRAIKEGIVKREDLVVVSKLWNSFHHPDNVRTAVERTLNDLQLDYLDLFYIHFPLAFKFVPLDEKYPPGFYTGKDNFAKEIIEEEPVPILDTYRALEKLVDEGLIKSLGISNFSGALIQDLLRGARIKPVALQIEHHPYLVQDRLITYAQKVGLQVVAYSSFGPLSFVELNNEKALHTKTLFENDTIKAIAQKHNVTPSHVLLKWSTQRGIAVIPKSSKKERLLENLKIEETFTLSDEEIKEINGLDQGLRFNDPWDWLGNEFPTFI

SEQ ID NO: 26 - protein, 329 aa, synthetic construct
  source 1..329: note = KlmXR C23H W24F
MTYLAPTVTLNNGSKMPLVGLGHFKIPNEVCAEQVYEAIKLGYRLFDGAQDYANEKEVGQGINRAIKEGIVKREDLVVVSKLWNSFHHPDNVRTAVERTLNDLQLDYLDLFYIHFPLAFKFVPLDEKYPPGFYTGKDNFAKEIIEEEPVPILDTYRALEKLVDEGLIKSLGISNFSGALIQDLLRGARIKPVALQIEHHPYLVQDRLITYAQKVGLQVVAYSSFGPLSFVELNNEKALHTKTLFENDTIKAIAQKHNVTPSHVLLKWSTQRGIAVIPKSSKKERLLENLKIEETFTLSDEEIKEINGLDQGLRFNDPWDWLGNEFPTFI

SEQ ID NO: 27 - protein, 329 aa, synthetic construct
  source 1..329: note = KlmXR C23Q W24F
MTYLAPTVTLNNGSKMPLVGLGQFKIPNEVCAEQVYEAIKLGYRLFDGAQDYANEKEVGQGINRAIKEGIVKREDLVVVSKLWNSFHHPDNVRTAVERTLNDLQLDYLDLFYIHFPLAFKFVPLDEKYPPGFYTGKDNFAKEIIEEEPVPILDTYRALEKLVDEGLIKSLGISNFSGALIQDLLRGARIKPVALQIEHHPYLVQDRLITYAQKVGLQVVAYSSFGPLSFVELNNEKALHTKTLFENDTIKAIAQKHNVTPSHVLLKWSTQRGIAVIPKSSKKERLLENLKIEETFTLSDEEIKEINGLDQGLRFNDPWDWLGNEFPTFI

SEQ ID NO: 28 - protein, 329 aa, synthetic construct
  source 1..329: note = KlmXR C23N W24F
MTYLAPTVTLNNGSKMPLVGLGNFKIPNEVCAEQVYEAIKLGYRLFDGAQDYANEKEVGQGINRAIKEGIVKREDLVVVSKLWNSFHHPDNVRTAVERTLNDLQLDYLDLFYIHFPLAFKFVPLDEKYPPGFYTGKDNFAKEIIEEEPVPILDTYRALEKLVDEGLIKSLGISNFSGALIQDLLRGARIKPVALQIEHHPYLVQDRLITYAQKVGLQVVAYSSFGPLSFVELNNEKALHTKTLFENDTIKAIAQKHNVTPSHVLLKWSTQRGIAVIPKSSKKERLLENLKIEETFTLSDEEIKEINGLDQGLRFNDPWDWLGNEFPTFI

SEQ ID NO: 29 - protein, 6 aa, synthetic construct
  source 1..6: note = Xylose reductase enzyme motif
  VARIANT 2: note = leucine or phenylalanine
GXGTFK

SEQ ID NO: 30 - protein, 6 aa, synthetic construct
  source 1..6: note = Xylose reductase enzyme motif
GYRLFD